European Patent Application EP 4 520 824 A1, published March 12, 2025. Title: DEOXYRIBOZYME THAT GENERATES FLUORESCENCE AND USES THEREOF. Applicant: Ustav organicke chemie a biochemie AV CR, v. v. i. Application EP. The sequence listing filed with the application follows.

SEQUENCE LISTING (60 sequences)

SEQ ID NO: 1 - DNA, 105 bp, synthetic construct
  source 1..105: mol_type = other DNA
ggaagagatggcgacgacacagggacgatgccgaatatcctcagtgcgcagggccgcaggggggagtgacttgggatggggggtccactaatgatctgcccgatg

SEQ ID NO: 2 - DNA, 20 bp, synthetic construct
  source 1..20: mol_type = other DNA
accgctcaggtgtagtatca

SEQ ID NO: 3 - DNA, 20 bp, synthetic construct
  source 1..20: mol_type = other DNA
catcgggcagatcattagtg

SEQ ID NO: 4 - DNA, 35 bp, synthetic construct
  source 1..35: mol_type = other DNA
gtcgccatctcttcctgatactacacctgagcggt

SEQ ID NO: 5 - DNA, 20 bp, synthetic construct
  source 1..20: mol_type = other DNA
  misc_feature 20: note = RNA
accgctcaggtgtagtatca

SEQ ID NO: 6 - DNA, 20 bp, synthetic construct
  source 1..20: mol_type = other DNA
catcgggcagatcattagtg

SEQ ID NO: 7 - DNA, 85 bp, synthetic construct
  source 1..85: mol_type = other DNA
ggaagagatgaccagggcagcgggacgctgacgaattttctcactatgtccgggacccgaggggcgtgaggagtgttgtgcaatt

SEQ ID NO: 8 - DNA, 47 bp, synthetic construct
  source 1..47: mol_type = other DNA
ggaagagatgactatgtccgggacccgaggggcgtgaggagtgttgt

SEQ ID NO: 9 - DNA, 105 bp, synthetic construct
  source 1..105: mol_type = other DNA
ggaagagatgaccagggcagcgggacgctgacgaattttctcactatgtccgggacccgaggggcgtgaggagtgttgtgcaattctcatgaactatccgctgga

SEQ ID NO: 10 - DNA, 20 bp, synthetic construct
  source 1..20: mol_type = other DNA
tccagcggatagttcatgag

SEQ ID NO: 11 - DNA, 20 bp, synthetic construct
  source 1..20: mol_type = other DNA
tccagcggatagttcatgag

SEQ ID NO: 12 - DNA, 85 bp, synthetic construct
  source 1..85: mol_type = other DNA
ggaagggatgagcagagtagcgcgacgatgacgaattttgtaactatgtccggttcctgtaaggcatgtggagtgttgtgcaatt

SEQ ID NO: 13 - DNA, 47 bp, synthetic construct
  source 1..47: mol_type = other DNA
ggaagggatgactatgtccggttcctgtaaggcatgtggagtgttgt

SEQ ID NO: 14 - DNA, 47 bp, synthetic construct
  source 1..47: mol_type = other DNA
ggaagggatgactatgcccggttcctgtaaggcatgtggggtgttgt

SEQ ID NO: 15 - DNA, 69 bp, synthetic construct
  source 1..69: mol_type = other DNA
ggaggrgatgratryryccggkhccrkwwyggcdtghggrgyryatyaacactaatgatctgcccgatg

SEQ ID NO: 16 - DNA, 69 bp, synthetic construct
  source 1..69: mol_type = other DNA
ggaagrgatgratryryccggkhccrkwwyggcdtghggrgyryttyaacactaatgatctgcccgatg

SEQ ID NO: 17 - DNA, 69 bp, synthetic construct
  source 1..69: mol_type = other DNA
ggaggrgatgrctryryccggkhccrkwwyggcdtghggrgyryagyaacactaatgatctgcccgatg

SEQ ID NO: 18 - DNA, 69 bp, synthetic construct
  source 1..69: mol_type = other DNA
ggaggrgatgratryryccggkhccykwwrggcdtghggrgyryatyaacactaatgatctgcccgatg

SEQ ID NO: 19 - DNA, 69 bp, synthetic construct
  source 1..69: mol_type = other DNA
ggaagrgatgrctryryccggkhccrkwwyggcdtghggrgyrytgyaacactaatgatctgcccgatg

SEQ ID NO: 20 - DNA, 69 bp, synthetic construct
  source 1..69: mol_type = other DNA
ggaagrgatgratryryccggkhccykwwrggcdtghggrgyryttyaacactaatgatctgcccgatg

SEQ ID NO: 21 - DNA, 69 bp, synthetic construct
  source 1..69: mol_type = other DNA
ggaggrgatgrctryryccggkhccykwwrggcdtghggrgyryagyaacactaatgatctgcccgatg

SEQ ID NO: 22 - DNA, 69 bp, synthetic construct
  source 1..69: mol_type = other DNA
ggaagrgatgrctryryccggkhccykwwrggcdtghggrgyrytgyaacactaatgatctgcccgatg

SEQ ID NO: 23 - DNA, 47 bp, synthetic construct
  source 1..47: mol_type = other DNA
ggaagggatgaatatgtccggttccagtatggcgtgtggagtgtttt

SEQ ID NO: 24 - DNA, 47 bp, synthetic construct
  source 1..47: mol_type = other DNA
ggaagggatgaatatgtccggttccagtatggcttgtggagtgtttt

SEQ ID NO: 25 - DNA, 77 bp, synthetic construct
  source 1..77: mol_type = other DNA
ggaagggatggaaggtcaatactatgtccggttcctgtaaggcatgtggagtgttgtattgaccttcattgaccttc

SEQ ID NO: 26 - DNA, 77 bp, synthetic construct
  source 1..77: mol_type = other DNA
ggaagggatggggcactgatactatgtccggttcctgtaaggcatgtggagtgttgtatcagtgcccagtgggcacg

SEQ ID NO: 27 - DNA, 77 bp, synthetic construct
  source 1..77: mol_type = other DNA
ggaagggatggatgatcggaactatgtccggttcctgtaaggcatgtggagtgttgttccgatcatccgaagatcag

SEQ ID NO: 28 - DNA, 77 bp, synthetic construct
  source 1..77: mol_type = other DNA
ggaagggatgaagtaatagcactatgtccggttcctgtaaggcatgtggagtgttgtgctattacttatctttccga

SEQ ID NO: 29 - DNA, 77 bp, synthetic construct
  source 1..77: mol_type = other DNA
ggaagggatgtaaaagataaactatgtccggttcctgtaaggcatgtggagtgttgtttatcttttattcgtgtgta

SEQ ID NO: 30 - DNA, 20 bp, synthetic construct
  source 1..20: mol_type = other DNA
gaaggtcaatgaaggtcaat

SEQ ID NO: 31 - DNA, 20 bp, synthetic construct
  source 1..20: mol_type = other DNA
cgtgcccactgggcactgat

SEQ ID NO: 32 - DNA, 20 bp, synthetic construct
  source 1..20: mol_type = other DNA
ctgatcttcggatgatcgga

SEQ ID NO: 33 - DNA, 20 bp, synthetic construct
  source 1..20: mol_type = other DNA
tcggaaagataagtaatagc

SEQ ID NO: 34 - DNA, 20 bp, synthetic construct
  source 1..20: mol_type = other DNA
tacacacgaataaaagataa

SEQ ID NO: 35 - DNA, 52 bp, synthetic construct
  source 1..52: mol_type = other DNA
  misc_feature 5: note = RNA
aaaacggaagggatgaatatgtccggttccttttaggcgtgtggagtgtttt

SEQ ID NO: 36 - DNA, 52 bp, synthetic construct
  source 1..52: mol_type = other DNA
  misc_feature 5: note = Uracil
aaaatggaagggatgaatatgtccggttccttttaggcgtgtggagtgtttt

SEQ ID NO: 37 - DNA, 47 bp, synthetic construct
  source 1..47: mol_type = other DNA
ggargddnnnnnnatryycggnnccnnnnnggsnnghgrrgygtdnn

SEQ ID NO: 38 - DNA, 85 bp, synthetic construct
  source 1..85: mol_type = other DNA
ggcagagatggcgctgtcatagggacagtgctacgcatgctcaccctctggggcaatcggggggcttcgacttgtatagagttag

SEQ ID NO: 39 - DNA, 50 bp, synthetic construct
  source 1..50: mol_type = other DNA
ggcagagatggcgcagccacgcatgctcaccctctggggcaatcgggggg

SEQ ID NO: 40 - DNA, 85 bp, synthetic construct
  source 1..85: mol_type = other DNA
ggcagagacggcggcgtcatagggacagtgctgtacatgctcaccctcaggggcaatcggggggcgtgaacttatatggagttac

SEQ ID NO: 41 - DNA, 50 bp, synthetic construct
  source 1..50: mol_type = other DNA
ggcagagacggcgcagctgtacatgctcaccctcaggggcaatcgggggg

SEQ ID NO: 42 - DNA, 105 bp, synthetic construct
  source 1..105: mol_type = other DNA
ggcagagacggcggcgtcatagggacagtgctgtacatgctcaccctcaggggcaatcggggggcgtgaacttatatggagttactaacactcttgacgagccgt

SEQ ID NO: 43 - DNA, 89 bp, synthetic construct
  source 1..89: mol_type = other DNA
ggcagagatggcgaaggtcaatgccacgcatgctcaccctctggggcaatcggggggattgaccttcattgaccttcgccatctctgcc

SEQ ID NO: 44 - DNA, 32 bp, synthetic construct
  source 1..32: mol_type = other DNA
ggcagagatggcgaaggtcaatgaaggtcaat

SEQ ID NO: 45 - DNA, 60 bp, synthetic construct
  source 1..60: mol_type = other DNA
  misc_feature 10: note = RNA
aaaaaaaaacggcagagatggcgcagccacgcatgctcaccctctggggcaatcgggggg

SEQ ID NO: 46 - DNA, 60 bp, synthetic construct
  source 1..60: mol_type = other DNA
  misc_feature 10: note = Uracil
aaaaaaaaatggcagagatggcgcagccacgcatgctcaccctctggggcaatcgggggg

SEQ ID NO: 47 - DNA, 12 bp, synthetic construct
  source 1..12: mol_type = other DNA
ggcagagahrgc

SEQ ID NO: 48 - DNA, 35 bp, synthetic construct
  source 1..35: mol_type = other DNA
kchdyrcatgctcmccckbdggggcaatcgggggg

SEQ ID NO: 49 - DNA, 39 bp, synthetic construct
  source 1..39: mol_type = other DNA
ggcagagayrcatgctcmccckbdggggcaatcgggggg

SEQ ID NO: 50 - DNA, 48 bp, synthetic construct
  source 1..48: mol_type = other DNA
ggcagagaggcgcagcccgcatgctcaccctctggggcaatcgggggg

SEQ ID NO: 51 - DNA, 46 bp, synthetic construct
  source 1..46: mol_type = other DNA
ggcagagagcgcagccgcatgctcaccctctggggcaatcgggggg

SEQ ID NO: 52 - DNA, 44 bp, synthetic construct
  source 1..44: mol_type = other DNA
ggcagagacgcagcgcatgctcaccctctggggcaatcgggggg

SEQ ID NO: 53 - DNA, 39 bp, synthetic construct
  source 1..39: mol_type = other DNA
ggcagagacgcatgctcaccctctggggcaatcgggggg

SEQ ID NO: 54 - DNA, 34 bp, synthetic construct
  source 1..34: mol_type = other DNA
ggcagcatgctcaccctctggggcaatcgggggg

SEQ ID NO: 55 - DNA, 105 bp, synthetic construct
  source 1..105: mol_type = other DNA
ggaagatatggcgcgaacaaatggacaatgccgaatatcccccgcacgcagggcaacaagggggagtgacttgggatgggggctgcactaatgatctgcccgatg

SEQ ID NO: 56 - DNA, 46 bp, synthetic construct
  source 1..46: mol_type = other DNA
ggaagaaaaagaatatccccaaaaggggagtgacttgggatggggg

SEQ ID NO: 57 - DNA, 46 bp, synthetic construct
  source 1..46: mol_type = other DNA
ggcagaaaaagaatatccccaaaaggggagtgacttgggatggggg

SEQ ID NO: 58 - DNA, 46 bp, synthetic construct
  source 1..46: mol_type = other DNA
ggaagaaaaagaatatccccaaaaggggagtgacttgcgatggggg

SEQ ID NO: 59 - DNA, 85 bp, synthetic construct
  source 1..85: mol_type = other DNA
ggcagagatggcaacgtcaacatgaggatgccgcatatccccagtgcacacttgggcagtggggagtgacttgggatgggggaaa

SEQ ID NO: 60 - DNA, 47 bp, synthetic construct
  source 1..47: mol_type = other DNA
ggaggagatggatatatccgggaccctatgggcgtgtggagcgtatc